European Patent Specification EP 4 232 021 B1, published May 27, 2026. Title: Sulfated C19 steroid hormones to treat and/or prevent proteotoxicity in protein-aggregation diseases. Applicant: Universidad Pablo de Olavide OTRI. The sequence listing filed with the application follows.

SEQUENCE LISTING (13 sequences)

SEQ ID NO: 1 - protein, 60 aa, Artificial Sequence
  Fig. 6 Sequence SUL-2
PNIVILMIDDLGYGDIASYGHPTQEYTQVDRMAAEGTRFTQAYSADSMCSPSRAGFITGR

SEQ ID NO: 2 - protein, 60 aa, Artificial Sequence
  Fig. 6 Sequence ARSC
PNIILVMADDLGIGDPGCYGNKTIRTPNIDRLASGGVKLTQHLAASPLCTPSRAAFMTGR

SEQ ID NO: 3 - protein, 60 aa, Artificial Sequence
  Fig. 6 Sequence ARSD
PNILLIMADDLGTGDLGCYGNNTLRTPNIDQLAEEGVRLTQHLAAAPLCTPSRAAFLTGR

SEQ ID NO: 4 - protein, 59 aa, Artificial Sequence
  Fig. 6 Sequence ARSE
PNILLLMADDLGIGDIGCYGNNTMRTPNIRLAEDGVKLTQHISAASLCTPSRAAFLTGR

SEQ ID NO: 5 - protein, 60 aa, Artificial Sequence
  Fig. 6 Sequence ARSH
PNIVLLMADDLGVGDLCCYGNNSVSTPNIDRLASEGVRLTQHLAAASMCTPSRAAFLTGR

SEQ ID NO: 6 - protein, 60 aa, Artificial Sequence
  Fig. 6 Sequence ARSF
PNIVLIMVDDLGIGDLGCYGNDTMRTPHIDRLAREGVRLTQHISAASLCSPSRSAFLTGR

SEQ ID NO: 7 - protein, 60 aa, Artificial Sequence
  Fig. 6 Sequence ARSG
PNFVIILADDMGWGDLGANWAETKDTANLDKMASEGMRFVDFHAAASTCSPSRASLLTGR

SEQ ID NO: 8 - protein, 60 aa, Artificial Sequence
  Fig. 6 Sequence ARSA
PNIVLIFADDLGYGDLGCYGHPSSTTPNLDQLAAGGLRFTDFYVPVSLCTPSRAALLTGR

SEQ ID NO: 9 - protein, 11 aa, Artificial Sequence
  Fig. 6 Sequence SUL-2_wormbase
SKRFRGSSKEA

SEQ ID NO: 10 - protein, 117 aa, Artificial Sequence
  Fig. 6 Sequence SUL-2_modified
SKRFRGSSIYGDSINEMSWAVGEVLDSLVNAGIAENTLVILMSDHGPHVELCLNGGSTAGLKGGKSNSYEGGFRIPFIAWQPGTVKPSRVSHEVISSMDLFPTFRGMQEQCLFEKEA

SEQ ID NO: 11 - protein, 120 aa, Artificial Sequence
  Fig. 6 Sequence SUL-2_curated
SKRFRGSSVRGIYGDSINEMSWAVGEVLDSLVNAGIAENTLVILMSDHGPHVELCLNGGSTAGLKGGKSNSYEGGFRIPFIAWQPGTVKPSRVSHEVISSMDLFPTFRGMQEQCLFEKEA

SEQ ID NO: 12 - protein, 120 aa, Artificial Sequence
  Fig. 6 Sequence CRE-SUL-2
SKRFRGSSVRGIYGDSINEMSWAVGEVLDSLVNAGIAENTLVILMSDHGPHVELCLNGGSTAGLKGGKSNSYEGGFRIPFIAWQPGTVKPSRVSHEVVSSMDLFPTFRAMNEECLFEKEA

SEQ ID NO: 13 - protein, 120 aa, Artificial Sequence
  Fig 6 Sequence CBR-SUL-2
SKRFRGSSVRGIYGDSINEMSWAVGEVLDSLVNAGIAENTLVILMSDHGPHVELCLNGGSTAGLKGGKSNSYEGGFRIPFIAWQPGTVKPSRVSHEVISSMDLFPTFRAMNEECLFEKEA